European Patent Application EP 4 733 318 A2, published April 29, 2026. Title: ANTIBODY AGAINST HUMAN IMMUNODEFICIENCY VIRUS TYPE 1 P24 AND TYPE 2 P26 AND USES THEREOF. Applicant: SHENZHEN MINDRAY BIO-MEDICAL ELECTRONICS CO., LTD. The sequence listing filed with the application follows.

SEQUENCE LISTING (42 sequences)

SEQ ID NO: 1 - protein, 8 aa, synthetic construct
GYTFISYW

SEQ ID NO: 2 - protein, 17 aa, synthetic construct
EIFPGSGHADYNEKFKD

SEQ ID NO: 3 - protein, 8 aa, synthetic construct
STTRRIDY

SEQ ID NO: 4 - protein, 11 aa, synthetic construct
RASGNIHNYLA

SEQ ID NO: 5 - protein, 7 aa, synthetic construct
NAITLAD

SEQ ID NO: 6 - protein, 9 aa, synthetic construct
QHFWSTPLT

SEQ ID NO: 7 - protein, 8 aa, synthetic construct
GFAFSTYD

SEQ ID NO: 8 - protein, 17 aa, synthetic construct
YISGGRGSTHYPDTVKG

SEQ ID NO: 9 - protein, 12 aa, synthetic construct
QRFSFGSSPFDV

SEQ ID NO: 10 - protein, 11 aa, synthetic construct
RTSENIYSFLA

SEQ ID NO: 11 - protein, 7 aa, synthetic construct
NVKTLAE

SEQ ID NO: 12 - protein, 9 aa, synthetic construct
QHHYGTPWT

SEQ ID NO: 13 - protein, 8 aa, synthetic construct
GFSLSNYG

SEQ ID NO: 14 - protein, 16 aa, synthetic construct
YIGADGRIYYANWAKS

SEQ ID NO: 15 - protein, 13 aa, synthetic construct
DMGTDAYGYATDI

SEQ ID NO: 16 - protein, 11 aa, synthetic construct
QASESIDIWLV

SEQ ID NO: 17 - protein, 7 aa, synthetic construct
DASKLAS

SEQ ID NO: 18 - protein, 12 aa, synthetic construct
QQGYTYSDIDNT

SEQ ID NO: 19 - protein, 8 aa, synthetic construct
GIDLSSNG

SEQ ID NO: 20 - protein, 16 aa, synthetic construct
FIKTTGNTYYASWAKG

SEQ ID NO: 21 - protein, 12 aa, synthetic construct
DPDYSYGYVLDP

SEQ ID NO: 22 - protein, 11 aa, synthetic construct
QASESIDIWFS

SEQ ID NO: 23 - protein, 7 aa, synthetic construct
DASKLAA

SEQ ID NO: 24 - protein, 12 aa, synthetic construct
QQGYSVSDVDNI

SEQ ID NO: 25 - protein, 9 aa, synthetic construct
GFTISSSYY

SEQ ID NO: 26 - protein, 18 aa, synthetic construct
CIYGGSSGSTSYASWAKG

SEQ ID NO: 27 - protein, 9 aa, synthetic construct
DRGDWYVDL

SEQ ID NO: 28 - protein, 11 aa, synthetic construct
QASQNIYNNLA

SEQ ID NO: 29 - protein, 7 aa, synthetic construct
RASTLES

SEQ ID NO: 30 - protein, 12 aa, synthetic construct
QGYAYSITTDYI

SEQ ID NO: 31 - protein, 8 aa, synthetic construct
GFDFSGVG

SEQ ID NO: 32 - protein, 17 aa, synthetic construct
YIYPKFGVRNYANSVKG

SEQ ID NO: 33 - protein, 12 aa, synthetic construct
AGYPGYGYYFDL

SEQ ID NO: 34 - protein, 11 aa, synthetic construct
QASQSIDSYLS

SEQ ID NO: 35 - protein, 7 aa, synthetic construct
GASTLES

SEQ ID NO: 36 - protein, 12 aa, synthetic construct
QGGYYSNSVIGA

SEQ ID NO: 37 - protein, 8 aa, synthetic construct
GFSLTSYN

SEQ ID NO: 38 - protein, 16 aa, synthetic construct
IVWSGGLIDYNSTLKS

SEQ ID NO: 39 - protein, 12 aa, synthetic construct
ENRHSHHDYFDY

SEQ ID NO: 40 - protein, 11 aa, synthetic construct
RASETVTTGVH

SEQ ID NO: 41 - protein, 7 aa, synthetic construct
GASNLES

SEQ ID NO: 42 - protein, 9 aa, synthetic construct
QQTWNDPLT